European Patent Application EP 4 239 073 A1, published September 6, 2023. Title: RECOMBINANT NUCLEIC ACID MOLECULE AND APPLICATION THEREOF IN PREPARATION OF CIRCULAR RNA. Applicant: Suzhou Curemed Biomedical Technology Co. Ltd. The sequence listing filed with the application follows.

SEQUENCE LISTING (80 sequences)

SEQ ID NO: 1 - DNA, 19 bp, synthetic construct
  misc_feature 1..19: note = sequence of PolyAC
  source 1..19: mol_type = other DNA
aaaaaacaaaaaacaaaac

SEQ ID NO: 2 - DNA, 1542 bp, synthetic construct
  misc_feature 1..1542: note = sequence of circular RNA
  source 1..1542: mol_type = other DNA
ggggttaaaacagcctgtgggttgatcccacccacagggcccactgggcgctagcactctggtatcacggtacctttgtgcgcctgttttatacttcctcccccaactgcaacttagaagtaacacaaaccgatcaacagtcagcgtggcacaccagccacgttttgatcaaacacttctgttaccccggactgagtatcaatagactgctcacgcggttgaaggagaaaacgttcgttatccggccaactacttcgagaaacctagtaacgccatggaagttgtggagtgtttcgctcagcactaccccagtgtagatcaggttgatgagtcaccgcattccccacgggtgaccgtggcggtggctgcgttggcggcctgcccatggggaaacccatgggacgctcttatacagacatggtgcgaagagtctattgagctagttggtagtcctccggcccctgaatgcggctaatcccaactgcggagcatacactctcaagccagagggtagtgtgtcgtaatgggcaactctgcagcggaaccgactactttgggtgtccgtgtttcattttattcctatactggctgcttatggtgacaattgagagattgttaccatatagctattggattggccatccggtgactaacagagctattatatatctttttgttgggtttataccacttagcttgaaagaggttaaaactctacattacattttaatactgaacaccgcaaaatggtgtcaaagggtgaggaattattcaccggcgtggtgcctatccttgtggaacttgatggagatgtgaacggacacaaattcagtgtatcaggagaaggagaaggagatgcaacatacggaaagctcactcttaaatttatctgcacaacaggaaagctcccggtgccttggcctacacttgtgacaacacttacatacggagtgcaatgcttctcgcgttaccctgatcacatgaaacaacacgatttcttcaagagtgcaatgcctgaaggatacgtgcaagaaagaacaatcttcttcaaggacgatggaaactacaagactcgtgcagaagtgaaatttgaaggagatacacttgtgaacagaatcgaacttaaaggaatcgatttcaaggaggatggaaacatccttggacacaaacttgaatacaactacaactcacacaacgtgtacatcatggcagataaacagaagaatggtatcaaagtgaactttaagattcgccacaacatcgaagatgggtctgtgcaacttgcagatcactaccaacagaatacgccgataggagatggacctgtgcttcttcctgataaccactacctttcaacacaatcagcactttcaaaggacccaaacgagaagcgagaccacatggtgcttcttgaatttgtgacagcagcaggaatcacacttggaatggatgaactttacaaatgaaaaaaacaaaaaacaaaacaaaaaacaaaaaacaaaacaaaaaacaaaaaacaaaaaaaaaacaaaaaacaaaacc

SEQ ID NO: 3 - protein, 238 aa, synthetic construct
  REGION 1..238: note = sequence of eGFP
MVSKGEELFTGVVPILVELDGDVNGHKFSVSGEGEGDATYGKLTLKFICTTGKLPVPWPTLVTTLTYGVQCFSRYPDHMKQHDFFKSAMPEGYVQERTIFFKDDGNYKTRAEVKFEGDTLVNRIELKGIDFKEDGNILGHKLEYNYNSHNVYIMADKQKNGIKVNFKIRHNIEDGSVQLADHYQQNTPIGDGPVLLPDNHYLSTQSALSKDPNEKRDHMVLLEFVTAAGILGMDELYK

SEQ ID NO: 4 - DNA, 222 bp, synthetic construct
  misc_feature 1..222: note = sequence of intron region II
  source 1..222: mol_type = other DNA
ggatcctaatacgactcactatagggagaccctcgcacagtgagcaactgacggaggttctacataaatgcctaacgactatccctttggggagtagggtcaagtgactcgaaacgatagacaacttgctttaacaagttggagatatagtctgctctgcatggtgacatgcagctggatataattccggggtaagattaacgaccttatctgaacataatg

SEQ ID NO: 5 - DNA, 128 bp, synthetic construct
  misc_feature 1..128: note = sequence of intron region I
  source 1..128: mol_type = other DNA
taattgaggcctgagtataaggtgacttatacttgtaatctatctaaacggggaacctctctagtagacaatcccgtgctaaattgtaggactaccgtcagttgctcactgtgcatcagatttctaga

SEQ ID NO: 6 - DNA, 163 bp, synthetic construct
  misc_feature 1..163: note = sequence of intron region II
  source 1..163: mol_type = other DNA
ctacataaatgcctaacgactatccctttggggagtagggtcaagtgactcgaaacgatagacaacttgctttaacaagttggagatatagtctgctctgcatggtgacatgcagctggatataattccggggtaagattaacgaccttatctgaacataatg

SEQ ID NO: 7 - DNA, 93 bp, synthetic construct
  misc_feature 1..93: note = sequence of intron region I
  source 1..93: mol_type = other DNA
taattgaggcctgagtataaggtgacttatacttgtaatctatctaaacggggaacctctctagtagacaatcccgtgctaaattgtaggact

SEQ ID NO: 8 - DNA, 59 bp, synthetic construct
  misc_feature 1..59: note = sequence of homology arm
  source 1..59: mol_type = other DNA
ggatcctaatacgactcactatagggagaccctcgcacagtgagcaactgacggaggtt

SEQ ID NO: 9 - DNA, 35 bp, synthetic construct
  misc_feature 1..35: note = sequence of homology arm
  source 1..35: mol_type = other DNA
accgtcagttgctcactgtgcatcagatttctaga

SEQ ID NO: 10 - DNA, 742 bp, synthetic construct
  misc_feature 1..742: note = sequence of Ev29 IRES
  source 1..742: mol_type = other DNA
ttaaaacagcctgtgggttgatcccacccacagggcccactgggcgctagcactctggtatcacggtacctttgtgcgcctgttttatacttcctcccccaactgcaacttagaagtaacacaaaccgatcaacagtcagcgtggcacaccagccacgttttgatcaaacacttctgttaccccggactgagtatcaatagactgctcacgcggttgaaggagaaaacgttcgttatccggccaactacttcgagaaacctagtaacgccatggaagttgtggagtgtttcgctcagcactaccccagtgtagatcaggttgatgagtcaccgcattccccacgggtgaccgtggcggtggctgcgttggcggcctgcccatggggaaacccatgggacgctcttatacagacatggtgcgaagagtctattgagctagttggtagtcctccggcccctgaatgcggctaatcccaactgcggagcatacactctcaagccagagggtagtgtgtcgtaatgggcaactctgcagcggaaccgactactttgggtgtccgtgtttcattttattcctatactggctgcttatggtgacaattgagagattgttaccatatagctattggattggccatccggtgactaacagagctattatatatctttttgttgggtttataccacttagcttgaaagaggttaaaactctacattacattttaatactgaacaccgcaaa

SEQ ID NO: 11 - DNA, 720 bp, synthetic construct
  misc_feature 1..720: note = sequence of eGFP
  source 1..720: mol_type = other DNA
atggtgtcaaagggtgaggaattattcaccggcgtggtgcctatccttgtggaacttgatggagatgtgaacggacacaaattcagtgtatcaggagaaggagaaggagatgcaacatacggaaagctcactcttaaatttatctgcacaacaggaaagctcccggtgccttggcctacacttgtgacaacacttacatacggagtgcaatgcttctcgcgttaccctgatcacatgaaacaacacgatttcttcaagagtgcaatgcctgaaggatacgtgcaagaaagaacaatcttcttcaaggacgatggaaactacaagactcgtgcagaagtgaaatttgaaggagatacacttgtgaacagaatcgaacttaaaggaatcgatttcaaggaggatggaaacatccttggacacaaacttgaatacaactacaactcacacaacgtgtacatcatggcagataaacagaagaatggtatcaaagtgaactttaagattcgccacaacatcgaagatggatcagtgcaacttgcagatcactaccaacagaatacgccgataggagatggacctgtgcttcttcctgataaccactacctttcaacacaatcagcactttcaaaggacccaaacgagaagcgagaccacatggtgcttcttgaatttgtgacagcagcaggaatcacacttggaatggatgaactttacaaatga

SEQ ID NO: 12 - DNA, 526 bp, synthetic construct
  misc_feature 1..526: note = sequence of truncated region I ofeGFP
  source 1..526: mol_type = other DNA
atggtgtcaaagggtgaggaattattcaccggcgtggtgcctatccttgtggaacttgatggagatgtgaacggacacaaattcagtgtatcaggagaaggagaaggagatgcaacatacggaaagctcactcttaaatttatctgcacaacaggaaagctcccggtgccttggcctacacttgtgacaacacttacatacggagtgcaatgcttctcgcgttaccctgatcacatgaaacaacacgatttcttcaagagtgcaatgcctgaaggatacgtgcaagaaagaacaatcttcttcaaggacgatggaaactacaagactcgtgcagaagtgaaatttgaaggagatacacttgtgaacagaatcgaacttaaaggaatcgatttcaaggaggatggaaacatccttggacacaaacttgaatacaactacaactcacacaacgtgtacatcatggcagataaacagaagaatggtatcaaagtgaactttaagattcgccacaacatcgaagatgggt

SEQ ID NO: 13 - DNA, 194 bp, synthetic construct
  misc_feature 1..194: note = sequence of truncated region II of eGFP
  source 1..194: mol_type = other DNA
ctgtgcaacttgcagatcactaccaacagaatacgccgataggagatggacctgtgcttcttcctgataaccactacctttcaacacaatcagcactttcaaaggacccaaacgagaagcgagaccacatggtgcttcttgaatttgtgacagcagcaggaatcacacttggaatggatgaactttacaaatga

SEQ ID NO: 14 - DNA, 4447 bp, synthetic construct
  misc_feature 1..4447: note = sequence of pUC57-EV29-eGFP
  source 1..4447: mol_type = other DNA
cgcgcgtttcggtgatgacggtgaaaacctctgacacatgcagctcccggagactgtcacagcttgtctgtaagcggatgccgggagcagacaagcccgtcagggcgcgtcagcgggtgttggcgggtgtcggggctggcttaactatgcggcatcagagcagattgtactgagagtgcaccatatgcggtgtgaaataccgcacagatgcgtaaggagaaaataccgcatcaggcgccattcgccattcaggctgcgcaactgttgggaagggcgatcggtgcgggcctcttcgctattacgccagctggcgaaagggggatgtgctgcaaggcgattaagttgggtaacgccagggttttcccagtcacgacgttgtaaaacgacggccagtgaattgacgcgtattgggatgaattcggatcctaatacgactcactatagggagaccctcgcacagtgagcaactgacggaggttctacataaatgcctaacgactatccctttggggagtagggtcaagtgactcgaaacgatagacaacttgctttaacaagttggagatatagtctgctctgcatggtgacatgcagctggatataattccggggtaagattaacgaccttatctgaacataatgctgtgcaacttgcagatcactaccaacagaatacgccgataggagatggacctgtgcttcttcctgataaccactacctttcaacacaatcagcactttcaaaggacccaaacgagaagcgagaccacatggtgcttcttgaatttgtgacagcagcaggaatcacacttggaatggatgaactttacaaatgaggggttaaaacagcctgtgggttgatcccacccacagggcccactgggcgctagcactctggtatcacggtacctttgtgcgcctgttttatacttcctcccccaactgcaacttagaagtaacacaaaccgatcaacagtcagcgtggcacaccagccacgttttgatcaaacacttctgttaccccggactgagtatcaatagactgctcacgcggttgaaggagaaaacgttcgttatccggccaactacttcgagaaacctagtaacgccatggaagttgtggagtgtttcgctcagcactaccccagtgtagatcaggttgatgagtcaccgcattccccacgggtgaccgtggcggtggctgcgttggcggcctgcccatggggaaacccatgggacgctcttatacagacatggtgcgaagagtctattgagctagttggtagtcctccggcccctgaatgcggctaatcccaactgcggagcatacactctcaagccagagggtagtgtgtcgtaatgggcaactctgcagcggaaccgactactttgggtgtccgtgtttcattttattcctatactggctgcttatggtgacaattgagagattgttaccatatagctattggattggccatccggtgactaacagagctattatatatctttttgttgggtttataccacttagcttgaaagaggttaaaactctacattacattttaatactgaacaccgcaaaatggtgtcaaagggtgaggaattattcaccggcgtggtgcctatccttgtggaacttgatggagatgtgaacggacacaaattcagtgtatcaggagaaggagaaggagatgcaacatacggaaagctcactcttaaatttatctgcacaacaggaaagctcccggtgccttggcctacacttgtgacaacacttacatacggagtgcaatgcttctcgcgttaccctgatcacatgaaacaacacgatttcttcaagagtgcaatgcctgaaggatacgtgcaagaaagaacaatcttcttcaaggacgatggaaactacaagactcgtgcagaagtgaaatttgaaggagatacacttgtgaacagaatcgaacttaaaggaatcgatttcaaggaggatggaaacatccttggacacaaacttgaatacaactacaactcacacaacgtgtacatcatggcagataaacagaagaatggtatcaaagtgaactttaagattcgccacaacatcgaagatgggttaattgaggcctgagtataaggtgacttatacttgtaatctatctaaacggggaacctctctagtagacaatcccgtgctaaattgtaggactaccgtcagttgctcactgtgcatcagatttctagaatcccaatggcgcgccgagcttggctcgagcatggtcatagctgtttcctgtgtgaaattgttatccgctcacaattccacacaacatacgagccggaagcataaagtgtaaagcctggggtgcctaatgagtgagctaactcacattaattgcgttgcgctcactgcccgctttccagtcgggaaacctgtcgtgccagctgcattaatgaatcggccaacgcgcggggagaggcggtttgcgtattgggcgctgttccgcttcctcgctcactgactcgctgcgctcggtcgttcggctgcggcgagcggtatcagctcactcaaaggcggtaatacggttatccacagaatcaggggataacgcaggaaagaacatgtgagcaaaaggccagcaaaaggccaggaaccgtaaaaaggccgcgttgctggcgtttttccataggctccgcccccctgacgagcatcacaaaaatcgacgctcaagtcagaggtggcgaaacccgacaggactataaagataccaggcgtttccccctggaagctccctcgtgcgctctcctgttccgaccctgccgcttaccggatacctgtccgcctttctcccttcgggaagcgtggcgctttctcatagctcacgctgtaggtatctcagttcggtgtaggtcgttcgctccaagctgggctgtgtgcacgaaccccccgttcagcccgaccgctgcgccttatccggtaactatcgtcttgagtccaacccggtaagacacgacttatcgccactggcagcagccactggtaacaggattagcagagcgaggtatgtaggcggtgctacagagttcttgaagtggtggcctaactacggctacactagaagaacagtatttggtatctgcgctctgctgaagccagttaccttcggaaaaagagttggtagctcttgatccggcaaacaaaccaccgctggtagcggtggtttttttgtttgcaagcagcagattacgcgcagaaaaaaaggatctcaagaagatcctttgatcttttctacggggtctgacgctcagtggaacgaaaactcacgttaagggattttggtcatgagattatcaaaaaggatcttcacctagatccttttaaattaaaaatgaagttttaaatcaatctaaagtatatatgagtaaacttggtctgacagttagaaaaactcatcgagcatcaaatgaaactgcaatttattcatatcaggattatcaataccatatttttgaaaaagccgtttctgtaatgaaggagaaaactcaccgaggcagttccataggatggcaagatcctggtatcggtctgcgattccgactcgtccaacatcaatacaacctattaatttcccctcgtcaaaaataaggttatcaagtgagaaatcaccatgagtgacgactgaatccggtgagaatggcaaaagtttatgcatttctttccagacttgttcaacaggccagccattacgctcgtcatcaaaatcactcgcatcaaccaaaccgttattcattcgtgattgcgcctgagcgaaacgaaatacgcgatcgctgttaaaaggacaattacaaacaggaatcgaatgcaaccggcgcaggaacactgccagcgcatcaacaatattttcacctgaatcaggatattcttctaatacctggaatgctgttttcccagggatcgcagtggtgagtaaccatgcatcatcaggagtacggataaaatgcttgatggtcggaagaggcataaattccgtcagccagtttagtctgaccatctcatctgtaacatcattggcaacgctacctttgccatgtttcagaaacaactctggcgcatcgggcttcccatacaatcgatagattgtcgcacctgattgcccgacattatcgcgagcccatttatacccatataaatcagcatccatgttggaatttaatcgcggcctagagcaagacgtttcccgttgaatatggctcatactcttcctttttcaatattattgaagcatttatcagggttattgtctcatgagcggatacatatttgaatgtatttagaaaaataaacaaataggggttccgcgcacatttccccgaaaagtgccacctgacgtctaagaaaccattattatcatgacattaacctataaaaataggcgtatcacgaggcccttttgtc

SEQ ID NO: 15 - DNA, 2494 bp, synthetic construct
  misc_feature 1..2494: note = sequence of truncatedregion I ofspCas9
  source 1..2494: mol_type = other DNA
atggactacaaggaccacgacggcgactacaaggaccacgacatcgactacaaggacgacgatgacaagatggcccccaagaagaagaggaaggtgggcatccacggcgtgcccgccgccgacaagaagtacagcatcggcctggacatcggcaccaacagcgtgggctgggccgtgatcaccgacgactacaaggtgcccagcaagaagttcaaggtgctgggcaacaccgacaggcacagcatcaagaagaacctgatcggcgccctgctgttcgacagcggcgagaccgccgaggccaccaggctgaagaggaccgccaggaggaggtacaccaggaggaagaacaggatctgctacctgcaggagatcttcagcaacgagatggccaaggtggacgacagcttcttccacaggctggaggagagcttcctggtggaggaggacaagaagcacgagaggcaccccatcttcggcaacatcgtggacgaggtggcctaccacgagaagtaccccaccatctaccacctgaggaagaagctggccgacagcaccgacaaggccgacctgaggctgatctacctggccctcgcccacatgatcaagttcaggggccacttcctgatcgagggcgacctgaaccccgacaacagcgacgtggacaagctgttcatccagctggtgcagacctacaaccagctgttcgaggagaaccccatcaacgccagcagggtggacgccaaggccatcctgagcgccaggctgagcaagagcaggaggctggagaacctgatcgcccagctgcccggcgagaagaagaacggcctgttcggcaacctgatcgccctgctgctgggcctgacccccaacttcaagagcaacttcgacctggccgaggacgccaagctgcagctgagcaaggacacctacgacgacgacctggacaacctgctggcccagatcggcgaccagtacgccgacctgttcctggccgccaagaacctgagcgacgccatcctgctgagcgacatcctgagggtgaacagcgagatcaccaaggcccccttgagcgccagcatgatcaagaggtacgacgagcaccaccaggacctgaccctgctgaaggccctggtgaggcagcagctgcccgagaagtacaaggagatcttcttcgaccagagcaagaacggctacgccggctacatcgacggcggcgccagccaggaggagttctacaagttcatcaagcccatcctggagaagatggacggcaccgaggagctgctggccaagctgaacagggaggacctgctgaggaagcagaggaccttcgacaacggcagcatcccccaccagatccacctgggcgagctgcacgccatcctgaggaggcaggaggacttctaccccttcctgaaggacaacagggagaagatcgagaagatcctgaccttcaggatcccctactacgtgggccccctggccaggggcaacagcaggttcgcctggatgaccaggaagagcgaggagaccatcaccccctggaacttcgaggaggtggtggacaagggcgccagcgcccagagcttcatcgagaggatgaccaacttcgacaagaacctgcccaacgagaaggtgctgcccaagcacagcctgctgtacgagtacttcaccgtgtacaacgagctgaccaaggtgaagtacgtgaccgagggcatgaggaagcccgccttcctgagcggcgagcagaagaaggccatcgtggacctgctgttcaagaccaacaggaaggtgaccgtgaagcagctgaaggaggactacttcaagaagatcgagtgcttcgacagcgtggagatcagcggcgtggaggacaggttcaacgccagcctgggcacctaccacgacctgctgaagatcatcaaggataaggacttcctggacaacgaggagaacgaggacatcctggaggacatcgtgctgaccctgacactgttcgaggacaaggagatgatcgaggagaggctgaagaagtacgcccacctgttcgacgacaaggtgatgaagcagctgaagaggaggaggtacaccggctggggcaggctgagcaggaagctgatcaacggcatcagggacaagcagagcggcaagaccatcctggacttcctgaagagcgacggcttcgccaacaggaacttcatgcagctgatccacgacgacagcctgaccttcaaggaggacatccagaaggcccaggtgagcggccagggcgacagcctgcacgagcacatcgccaacctggccggcagccccgccatcaagaagggcatcctgcagaccgtgaaggtggtggacgagctggtgaaggtgatgggcaggcacaagcccgagaacatcgtgatcgagatggccagggagaaccagaccacccagaagggccagaagaacagcagggagaggatgaagaggatcgaggagggcatcaaggagcttgggt

SEQ ID NO: 16 - DNA, 1766 bp, synthetic construct
  misc_feature 1..1766: note = sequence of truncatedregion II ofspCas9
  source 1..1766: mol_type = other DNA
ctgacatcctgaaggagtaccccgtggagaacacccagctgcagaacgagaagctgtacctctactacctgcagaacggcagggacatgtacgtggaccaggagctggacatcaacaggctgagcgactacgacgtggaccacatcgtgccccagagcttcctgaaggacgacagcatcgacaacaaggtgctgaccaggagcgacaagaacaggggcaagagcgacaacgtgcccagcgaggaggtggtgaagaagatgaagaactactggaagcagctgctgaacgccaagctgatcacccagaggaagttcgacaacctgaccaaggccgagaggggcggcctgagcgagctggacaaggccggcttcatcaagaggcagctggtggagaccaggcagatcaccaagcacgtggcccagatcctggacagcaggatgaacaccaagtacgacgagaacgacaagctgatcagggaggtgagggtgatcaccctgaagagcaagctggtgagcgacttcaggaaggacttccagttctacaaggtgagggagatcaacaactaccaccacgcccacgacgcctacctgaacgccgtggtgggcaccgccctgatcaagaagtaccccaagctggagagcgagttcgtgtacggcgactacaaggtgtacgacgtgagaaagatgatcgccaagagcgagcaggagatcggcaaggccaccgccaagtacttcttctacagcaacatcatgaacttcttcaagaccgagatcaccctggccaacggcgagatcaggaagaggcccctgatcgagaccaacggcgagaccggcgagatcgtgtgggacaagggcagggacttcgccaccgtgaggaaggtgctgagcatgccccaggtgaacatcgtgaagaagaccgaggtgcagaccggcggcttcagcaaggagagcatcctgcccaagaggaacagcgacaagctgatcgccaggaagaaggactgggaccccaagaagtacggcggcttcgacagccccaccgtggcctacagcgtgctggtggtggccaaggtggagaagggcaagagcaaaaagctgaagagcgtgaaggagctgctgggcatcaccatcatggagaggagcagcttcgagaagaaccccatcgacttcctggaggccaagggctacaaggaggtgaggaaggacctgatcatcaagctgcccaagtacagcctgttcgagctggagaacggcaggaagaggatgctggccagcgccggcgagctgcagaagggcaacgagctggccctgcccagcaagtacgtgaacttcctgtacctggccagccactacgagaagctgaagggcagccccgaggacaacgagcagaagcagctgttcgtggagcagcacaagcactacctggacgagatcatcgagcagatcagcgagttcagcaagagggtgatcctggccgacgccaacctggacaaggtgctgagcgcctacaacaagcacagggacaagcccatcagggagcaggccgagaacatcatccacctgttcaccctgaccaacctgggcgcccccgccgccttcaagtacttcgacaccaccatcgacaggaagaggtacaccagcaccaaggaggtgctggacgccaccctgatccaccagagcatcaccggcctgtacgagaccaggatcgacctgagccagctgggcggcgactccggccctcccaagaagaagaggaaggtgggcggctga

SEQ ID NO: 17 - DNA, 826 bp, synthetic construct
  misc_feature 1..826: note = sequence of truncatedregion I offLUC
  source 1..826: mol_type = other DNA
atggaggacgccaagaacatcaagaagggccctgcccctttctaccctctggaggacggcaccgccggcgagcagctgcacaaggccatgaagaggtacgccctggtgcctggcaccatcgccttcaccgacgcccacatcgaggtggacatcacctacgccgagtacttcgagatgagcgtgaggctggccgaggccatgaagaggtacggcctgaacaccaaccacaggatcgtggtgtgcagcgagaacagcctgcagttcttcatgcctgtgctgggcgccctgttcatcggcgtggccgtggcccctgccaacgacatctacaacgagagggagctgctgaacagcatgggcatcagccagcctaccgtggtgttcgtgagcaagaagggcctgcagaagatcctgaacgtgcagaagaagctgcctatcatccagaagatcatcatcatggacagcaagaccgactaccagggcttccagagcatgtacaccttcgtgaccagccacctgcctcctggcttcaacgagtacgacttcgtgcctgagagcttcgacagggacaagaccatcgccctgatcatgaacagcagcggcagcaccggcctgcctaagggcgtggccctgcctcacaggaccgcctgcgtgaggttcagccacgccagggaccctatcttcggcaaccagatcatccctgacaccgccatcctgagcgtggtgcctttccaccacggcttcggcatgttcaccaccctgggctacctgatctgcggcttcagggtggtgctgatgtacaggttcgaggaggagctgttccttaggt

SEQ ID NO: 18 - DNA, 827 bp, synthetic construct
  misc_feature 1..827: note = sequence of truncatedregion II offLUC
  source 1..827: mol_type = other DNA
ctctgcaggactacaagatccagagcgccctgctggtgcctaccctgttcagcttcttcgccaagagcaccctgatcgacaagtacgacctgagcaacctgcacgagatcgccagcggcggcgcccctctgagcaaggaggtgggcgaggccgtggccaagaggttccacctgcctggcatcaggcagggctacggcctgaccgagaccaccagcgccatcctgatcacccctgagggcgacgacaagcctggcgccgtgggcaaggtggtgcctttcttcgaggccaaggtggtggacctggacaccggcaagaccctgggcgtgaaccagaggggcgagctgtgcgtgaggggccctatgatcatgagcggctacgtgaacaaccctgaggccaccaacgccctgatcgacaaggacggctggctgcacagcggcgacatcgcctactgggacgaggacgagcacttcttcatcgtggacaggctgaagagcctgatcaagtacaagggctaccaggtggcccctgccgagctggagagcatcctgctgcagcaccctaacatcttcgacgccggcgtggctggcttgcctgatgacgatgctggagagctgcctgccgccgtggtggtgctggagcacggcaagaccatgaccgagaaggagatcgtggactacgtggccagccaggtgaccaccgccaagaagctgaggggcggcgtggtgttcgtggacgaggtgcctaagggcctgaccggcaagctggacgccaggaagatcagggagatcctgatcaaggccaagaagggcggcaagatcgccgtgtga

SEQ ID NO: 19 - DNA, 1351 bp, synthetic construct
  misc_feature 1..1351: note = sequence of truncatedregion I ofIL12
  source 1..1351: mol_type = other DNA
atgagggtgaccgcccctaggaccctgatcctgctgctgagcggcgccctggccctcaccgagacctgggccggcagcggaagcatgtgggagctggagaaggacgtgtacgtggtggaggtcgactggacccctgacgcccctggcgagaccgtgaacctgacctgcgacacccctgaggaggacgacatcacctggaccagcgaccagaggcacggcgtgatcggcagcggcaagaccctgaccatcaccgtgaaggagttcctggacgccggccagtacacctgccacaagggcggcgagaccctgagccactcccacctgctgctgcacaagaaggagaacggcatctggagcaccgagatcctgaagaacttcaagaacaagaccttcctgaagtgcgaggcccctaactacagcggcaggttcacctgcagctggctggtgcagaggaacatggacctgaagttcaacatcaagagcagcagctccagccctgacagcagggccgtgacctgcggcatggccagcctgagcgccgagaaggtgaccctggaccagagggactacgagaagtacagcgtgagctgccaggaggacgtgacctgccctaccgccgaggagaccctgcctatcgagctggccctggaggccaggcagcagaacaagtacgagaactacagcaccagcttcttcatcagggacatcatcaagcctgaccctcctaagaacctgcagatgaagcctctgaagaacagccaggtggaggtgagctgggagtaccctgacagctggagcacccctcacagctacttcagcctgaagttcttcgtgaggatccagaggaagaaggagaagatgaaggagaccgaggagggctgcaaccagaagggcgccttcctggtggagaagaccagcaccgaggtgcagtgcaagggcggcaacgtgtgcgtgcaggcccaggacaggtactacaacagcagctgcagcaagtgggcctgcgtgccttgcagggtgaggagcgtgcctggcgtgggcgtccctggcgtgggcagggtgatccctgtgagcggccctgccaggtgcctgagccagagcaggaacctgctgaagaccaccgacgacatggtgaagaccgccagggagaagctgaagcactacagctgcaccgccgaggacatcgaccacgaggacatcaccagggaccagaccagcaccctgaagacctgcctgcctctggagctgcacaagaacgagagctgcctggccaccagggagaccagcagcaccaccaggggcagctgcctgcctcctcagaagaccagcctgatgatgaccctgtgccttgggt

SEQ ID NO: 20 - DNA, 284 bp, synthetic construct
  misc_feature 1..284: note = sequence of truncatedregion II ofIL12
  source 1..284: mol_type = other DNA
ctatctacgaggacctgaagatgtaccagaccgagttccaggccatcaacgccgccctgcagaaccacaatcaccagcagatcatcctggacaagggcatgctggtggccatcgacgagctgatgcagagcctgaaccacaacggcgagaccctgaggcagaagcctcctgtgggcgaggccgacccttacagggtgaagatgaagctgtgcatcctgctgcacgccttcagcaccagggtggtgaccatcaacagggtgatgggctacctgagcagcgcctga

SEQ ID NO: 21 - DNA, 699 bp, synthetic construct
  misc_feature 1..699: note = sequence of truncatedregion I ofFLAG-con1-SPOP167-274
  source 1..699: mol_type = other DNA
atggactacaaggacgacgacgataaggccagcagcgccgtgctgcagaagaagatcaccgactacttccaccccaagaagggcagcggctctggcagcggaagcgtgaacatcagcggccagaacaccatgaacatggtgaaggtgcccgagtgcagactggccgacgagctgggcggcctgtgggagaacagcaggttcaccgactgctgcctgtgcgtggccggccaggagttccaggcccacaaggccatcctggccgccaggagccccgtgttcagcgccatgttcgagcacgagatggaggagagcaagaagaacagagtggagatcaacgacgtggagcccgaggtgttcaaggagatgatgtgcttcatctacaccggcaaggcccccaacctggacaagatggccgacgacctgctggccgccgccgacaagtacgccctggagagactgaaggtgatgtgcgaggacgccctgtgcagcaacctgagcgtggagaacgccgccgagatcctcatcctggccgacctgcacagcgccgaccagctgaagacccaggccgtggacttcatcaactaccacgccagcgacgtgctggagaccagcggctggaagagcatggtggtgagccacccccacctggtggccgaggcctacaggagcctggccagcgcccagtgccccttcttgggt

SEQ ID NO: 22 - DNA, 30 bp, synthetic construct
  misc_feature 1..30: note = sequence of truncatedregion II ofFLAG-con1-SPOP167-274
  source 1..30: mol_type = other DNA
cctcccaggaagagactgaagcagagctga

SEQ ID NO: 23 - DNA, 20 bp, synthetic construct
  misc_feature 1..20: note = primer sequence
  source 1..20: mol_type = other DNA
tacttgtcgatcagggtgct

SEQ ID NO: 24 - DNA, 20 bp, synthetic construct
  misc_feature 1..20: note = primer sequence
  source 1..20: mol_type = other DNA
tggacagcaagaccgactac

SEQ ID NO: 25 - DNA, 20 bp, synthetic construct
  misc_feature 1..20: note = primer sequence
  source 1..20: mol_type = other DNA
ctgcatcagctcgtcgatgg

SEQ ID NO: 26 - DNA, 22 bp, synthetic construct
  misc_feature 1..22: note = primer sequence
  source 1..22: mol_type = other DNA
tactacaacagcagctgcagca

SEQ ID NO: 27 - DNA, 754 bp, synthetic construct
  misc_feature 1..754: note = sequence of truncatedregion II ofFLAG-con1-SPOP167-274
  source 1..754: mol_type = other DNA
ctttaccgacaagaccagcgccaccgtgatctgcaggaagaacgccagcatcagcgtgagggcccaggacaggtactacagcagcagctggagcgagtgggccagcgtgccctgcagcggcagcagcggcggcgggggcagccccggcggcggcagcagcaggaacctgcccgtggccacccctgatcccggaatgttcccttgcctgcaccacagccagaacctgctgagggccgtgagcaacatgctgcagaaggccaggcagaccctggagttctacccctgcaccagcgaggagatcgaccacgaggacatcaccaaggacaagaccagcaccgtggaggcctgtctgcccttggagctgaccaagaacgagagctgcctgaacagcagggagaccagcttcatcaccaacggcagctgcctggccagcaggaagaccagcttcatgatggccctgtgcctgagcagcatctacgaggacctgaagatgtaccaggtggagttcaagaccatgaacgccaagctgctgatggaccccaagaggcagatcttcctggaccagaacatgctggccgtgatcgacgagctgatgcaggccctgaacttcaacagcgagaccgtgccccagaagagcagcctggaggagcccgacttctacaagaccaagatcaagctgtgcatcctgctgcacgccttcaggatcagagccgtgaccatcgacagggtgatgagctacctgaacgccagctga

SEQ ID NO: 28 - DNA, 866 bp, synthetic construct
  misc_feature 1..866: note = sequence of truncatedregion I ofFLAG-con1-SPOP167-274
  source 1..866: mol_type = other DNA
atgtgccaccagcagctggtgatcagctggttcagcctggtgttcctggccagccccctggtggccatctgggagctgaagaaggacgtgtacgtggtggagctggactggtaccccgacgcccccggcgagatggtggtgctgacctgcgacacccccgaggaggacggcatcacctggaccctggaccagagcagcgaggtgctgggcagcggcaagaccctgaccatccaggtgaaggagttcggcgacgccggccagtacacctgccacaagggcggcgaggtgctgagccacagcctgctgctgctccacaagaaggaggacggcatctggagcaccgacatcctgaaggaccagaaggagcccaagaacaagaccttcctgaggtgcgaggccaagaactacagcggcaggttcacctgctggtggctgaccaccatcagcaccgacctgaccttcagcgtgaagagcagcaggggcagcagcgacccccagggcgtgacctgcggcgctgccacattgtctgctgaaagggttagaggcgacaacaaggagtacgaatacagcgtggagtgccaggaggacagcgcctgccccgccgccgaggagagcctgcccatcgaggtgatggtggacgccgtgcacaagctgaagtacgagaactacaccagcagcttcttcatcagggacatcatcaagcccgaccctcccaagaacctgcagctgaagcccctgaagaacagcaggcaggtggaggtgagctgggagtaccccgacacctggagcacccctcacagctacttcagcctgaccttctgcgtgcaggtccagggcaagagcaagcgggagaagaaggatcgggt

SEQ ID NO: 29 - DNA, 1283 bp, synthetic construct
  misc_feature 1..1283: note = sequence of truncatedregion II ofFLAG-con1-SPOP167-274
  source 1..1283: mol_type = other DNA
ctaccgacatcctgaaggaccagaaggagcccaagaacaagaccttcctgaggtgcgaggccaagaactacagcggcaggttcacctgctggtggctgaccaccatcagcaccgacctgaccttcagcgtgaagagcagcaggggcagcagcgacccccagggcgtgacctgcggcgctgccacattgtctgctgaaagggttagaggcgacaacaaggagtacgaatacagcgtggagtgccaggaggacagcgcctgccccgccgccgaggagagcctgcccatcgaggtgatggtggacgccgtgcacaagctgaagtacgagaactacaccagcagcttcttcatcagggacatcatcaagcccgaccctcccaagaacctgcagctgaagcccctgaagaacagcaggcaggtggaggtgagctgggagtaccccgacacctggagcacccctcacagctacttcagcctgaccttctgcgtgcaggtccagggcaagagcaagcgggagaagaaggacagggtgttcaccgacaagaccagcgccaccgtgatctgcaggaagaacgccagcatcagcgtgagggcccaggacaggtactacagcagcagctggagcgagtgggccagcgtgccctgcagcggcagcagcggcggcgggggcagccccggcggcggcagcagcaggaacctgcccgtggccacccctgatcccggaatgttcccttgcctgcaccacagccagaacctgctgagggccgtgagcaacatgctgcagaaggccaggcagaccctggagttctacccctgcaccagcgaggagatcgaccacgaggacatcaccaaggacaagaccagcaccgtggaggcctgtctgcccttggagctgaccaagaacgagagctgcctgaacagcagggagaccagcttcatcaccaacggcagctgcctggccagcaggaagaccagcttcatgatggccctgtgcctgagcagcatctacgaggacctgaagatgtaccaggtggagttcaagaccatgaacgccaagctgctgatggaccccaagaggcagatcttcctggaccagaacatgctggccgtgatcgacgagctgatgcaggccctgaacttcaacagcgagaccgtgccccagaagagcagcctggaggagcccgacttctacaagaccaagatcaagctgtgcatcctgctgcacgccttcaggatcagagccgtgaccatcgacagggtgatgagctacctgaacgccagctga

SEQ ID NO: 30 - DNA, 337 bp, synthetic construct
  misc_feature 1..337: note = sequence of truncatedregion I ofFLAG-con1-SPOP167-274
  source 1..337: mol_type = other DNA
atgtgccaccagcagctggtgatcagctggttcagcctggtgttcctggccagccccctggtggccatctgggagctgaagaaggacgtgtacgtggtggagctggactggtaccccgacgcccccggcgagatggtggtgctgacctgcgacacccccgaggaggacggcatcacctggaccctggaccagagcagcgaggtgctgggcagcggcaagaccctgaccatccaggtgaaggagttcggcgacgccggccagtacacctgccacaagggcggcgaggtgctgagccacagcctgctgctgctccacaagaaggaggacggcatttggt

SEQ ID NO: 31 - DNA, 599 bp, synthetic construct
  misc_feature 1..599: note = sequence of truncatedregion II ofFLAG-con1-SPOP167-274
  source 1..599: mol_type = other DNA
ctagcaggaacctgcccgtggccacccctgatcccggaatgttcccttgcctgcaccacagccagaacctgctgagggccgtgagcaacatgctgcagaaggccaggcagaccctggagttctacccctgcaccagcgaggagatcgaccacgaggacatcaccaaggacaagaccagcaccgtggaggcctgtctgcccttggagctgaccaagaacgagagctgcctgaacagcagggagaccagcttcatcaccaacggcagctgcctggccagcaggaagaccagcttcatgatggccctgtgcctgagcagcatctacgaggacctgaagatgtaccaggtggagttcaagaccatgaacgccaagctgctgatggaccccaagaggcagatcttcctggaccagaacatgctggccgtgatcgacgagctgatgcaggccctgaacttcaacagcgagaccgtgccccagaagagcagcctggaggagcccgacttctacaagaccaagatcaagctgtgcatcctgctgcacgccttcaggatcagagccgtgaccatcgacagggtgatgagctacctgaacgccagctga

SEQ ID NO: 32 - DNA, 1021 bp, synthetic construct
  misc_feature 1..1021: note = sequence of truncatedregion I ofFLAG-con1-SPOP167-274
  source 1..1021: mol_type = other DNA
atgtgccaccagcagctggtgatcagctggttcagcctggtgttcctggccagccccctggtggccatctgggagctgaagaaggacgtgtacgtggtggagctggactggtaccccgacgcccccggcgagatggtggtgctgacctgcgacacccccgaggaggacggcatcacctggaccctggaccagagcagcgaggtgctgggcagcggcaagaccctgaccatccaggtgaaggagttcggcgacgccggccagtacacctgccacaagggcggcgaggtgctgagccacagcctgctgctgctccacaagaaggaggacggcatctggagcaccgacatcctgaaggaccagaaggagcccaagaacaagaccttcctgaggtgcgaggccaagaactacagcggcaggttcacctgctggtggctgaccaccatcagcaccgacctgaccttcagcgtgaagagcagcaggggcagcagcgacccccagggcgtgacctgcggcgctgccacattgtctgctgaaagggttagaggcgacaacaaggagtacgaatacagcgtggagtgccaggaggacagcgcctgccccgccgccgaggagagcctgcccatcgaggtgatggtggacgccgtgcacaagctgaagtacgagaactacaccagcagcttcttcatcagggacatcatcaagcccgaccctcccaagaacctgcagctgaagcccctgaagaacagcaggcaggtggaggtgagctgggagtaccccgacacctggagcacccctcacagctacttcagcctgaccttctgcgtgcaggtccagggcaagagcaagcgggagaagaaggacagggtgttcaccgacaagaccagcgccaccgtgatctgcaggaagaacgccagcatcagcgtgagggcccaggacaggtactacagcagcagctggagcgagtgggccagcgtgccctgcagcggcagcagcggcggcgggggcagccccggcggtgggt

SEQ ID NO: 33 - DNA, 335 bp, synthetic construct
  misc_feature 1..335: note = sequence of truncatedregion II ofFLAG-con1-SPOP167-274
  source 1..335: mol_type = other DNA
cttgcctggccagcaggaagaccagcttcatgatggccctgtgcctgagcagcatctacgaggacctgaagatgtaccaggtggagttcaagaccatgaacgccaagctgctgatggaccccaagaggcagatcttcctggaccagaacatgctggccgtgatcgacgagctgatgcaggccctgaacttcaacagcgagaccgtgccccagaagagcagcctggaggagcccgacttctacaagaccaagatcaagctgtgcatcctgctgcacgccttcaggatcagagccgtgaccatcgacagggtgatgagctacctgaacgccagctga

SEQ ID NO: 34 - DNA, 1285 bp, synthetic construct
  misc_feature 1..1285: note = sequence of truncatedregion I ofFLAG-con1-SPOP167-274
  source 1..1285: mol_type = other DNA
atgtgccaccagcagctggtgatcagctggttcagcctggtgttcctggccagccccctggtggccatctgggagctgaagaaggacgtgtacgtggtggagctggactggtaccccgacgcccccggcgagatggtggtgctgacctgcgacacccccgaggaggacggcatcacctggaccctggaccagagcagcgaggtgctgggcagcggcaagaccctgaccatccaggtgaaggagttcggcgacgccggccagtacacctgccacaagggcggcgaggtgctgagccacagcctgctgctgctccacaagaaggaggacggcatctggagcaccgacatcctgaaggaccagaaggagcccaagaacaagaccttcctgaggtgcgaggccaagaactacagcggcaggttcacctgctggtggctgaccaccatcagcaccgacctgaccttcagcgtgaagagcagcaggggcagcagcgacccccagggcgtgacctgcggcgctgccacattgtctgctgaaagggttagaggcgacaacaaggagtacgaatacagcgtggagtgccaggaggacagcgcctgccccgccgccgaggagagcctgcccatcgaggtgatggtggacgccgtgcacaagctgaagtacgagaactacaccagcagcttcttcatcagggacatcatcaagcccgaccctcccaagaacctgcagctgaagcccctgaagaacagcaggcaggtggaggtgagctgggagtaccccgacacctggagcacccctcacagctacttcagcctgaccttctgcgtgcaggtccagggcaagagcaagcgggagaagaaggacagggtgttcaccgacaagaccagcgccaccgtgatctgcaggaagaacgccagcatcagcgtgagggcccaggacaggtactacagcagcagctggagcgagtgggccagcgtgccctgcagcggcagcagcggcggcgggggcagccccggcggcggcagcagcaggaacctgcccgtggccacccctgatcccggaatgttcccttgcctgcaccacagccagaacctgctgagggccgtgagcaacatgctgcagaaggccaggcagaccctggagttctacccctgcaccagcgaggagatcgaccacgaggacatcaccaaggacaagaccagcaccgtggaggcctgtctgcccttggagctgaccaagaacgagagctgcctgaacagcagggagaccagcttcatcaccaatgggt

SEQ ID NO: 35 - DNA, 1409 bp, synthetic construct
  misc_feature 1..1409: note = sequence of truncatedregion II ofFLAG-con1-SPOP167-274
  source 1..1409: mol_type = other DNA
ctggcaagaccctgaccatccaggtgaaggagttcggcgacgccggccagtacacctgccacaagggcggcgaggtgctgagccacagcctgctgctgctccacaagaaggaggacggcatctggagcaccgacatcctgaaggaccagaaggagcccaagaacaagaccttcctgaggtgcgaggccaagaactacagcggcaggttcacctgctggtggctgaccaccatcagcaccgacctgaccttcagcgtgaagagcagcaggggcagcagcgacccccagggcgtgacctgcggcgctgccacattgtctgctgaaagggttagaggcgacaacaaggagtacgaatacagcgtggagtgccaggaggacagcgcctgccccgccgccgaggagagcctgcccatcgaggtgatggtggacgccgtgcacaagctgaagtacgagaactacaccagcagcttcttcatcagggacatcatcaagcccgaccctcccaagaacctgcagctgaagcccctgaagaacagcaggcaggtggaggtgagctgggagtaccccgacacctggagcacccctcacagctacttcagcctgaccttctgcgtgcaggtccagggcaagagcaagcgggagaagaaggacagggtgttcaccgacaagaccagcgccaccgtgatctgcaggaagaacgccagcatcagcgtgagggcccaggacaggtactacagcagcagctggagcgagtgggccagcgtgccctgcagcggcagcagcggcggcgggggcagccccggcggcggcagcagcaggaacctgcccgtggccacccctgatcccggaatgttcccttgcctgcaccacagccagaacctgctgagggccgtgagcaacatgctgcagaaggccaggcagaccctggagttctacccctgcaccagcgaggagatcgaccacgaggacatcaccaaggacaagaccagcaccgtggaggcctgtctgcccttggagctgaccaagaacgagagctgcctgaacagcagggagaccagcttcatcaccaacggcagctgcctggccagcaggaagaccagcttcatgatggccctgtgcctgagcagcatctacgaggacctgaagatgtaccaggtggagttcaagaccatgaacgccaagctgctgatggaccccaagaggcagatcttcctggaccagaacatgctggccgtgatcgacgagctgatgcaggccctgaacttcaacagcgagaccgtgccccagaagagcagcctggaggagcccgacttctacaagaccaagatcaagctgtgcatcctgctgcacgccttcaggatcagagccgtgaccatcgacagggtgatgagctacctgaacgccagctga

SEQ ID NO: 36 - DNA, 211 bp, synthetic construct
  misc_feature 1..211: note = sequence of truncatedregion I ofFLAG-con1-SPOP167-274
  source 1..211: mol_type = other DNA
atgtgccaccagcagctggtgatcagctggttcagcctggtgttcctggccagccccctggtggccatctgggagctgaagaaggacgtgtacgtggtggagctggactggtaccccgacgcccccggcgagatggtggtgctgacctgcgacacccccgaggaggacggcatcacctggaccctggaccagagcagcgaggtgcttgggt

SEQ ID NO: 37 - RNA, 60 nt, synthetic construct
  misc_feature 1..60: note = sequence of S1m
  source 1..60: mol_type = other RNA
atgcggccgccgaccagaatcatgcaagtgcgtaagatagtcgcgggtcggcggccgcat

SEQ ID NO: 38 - DNA, 1464 bp, synthetic construct
  misc_feature 1..1464: note = sequence of circular RNA
  source 1..1464: mol_type = other DNA
ctgtgcaacttgcagatcactaccaacagaatacgccgataggagatggacctgtgcttcttcctgataaccactacctttcaacacaatcagcactttcaaaggacccaaacgagaagcgagaccacatggtgcttcttgaatttgtgacagcagcaggaatcacacttggaatggatgaactttacaaatgaggttataacagcctgtgggttgatcccacccacagggcccactgggcgctagcactctggtatcacggtacctttgtgcgcctgttttatacttcctcccccaactgcaacttagaagtaacacaaaccgatcaacagtcagcgtggcacaccagccacgttttgatcaaacacttctgttaccccggactgagtatcaatagactgctcacgcggttgaaggagaaaacgttcgttatccggccaactacttcgagaaacctagtaacgccatggaagttgtggagtgtttcgctcagcactaccccagtgttgatcaggttgttgagtcaccgcattccccacgggtgtccgtggcggtggctgcgttggcggcctgcccatggggaaacccatgggacgctcttatacagacatggtgcgaagagtctattgagcttgttggtagtcctccggcccctgaatgcggctaatcccaactgcggagcatacactctcaagccagagggtagtgtgtcgtattgggcaactctgcagcggaaccgactactttgggtgtccgtgtttcattttattcctatactggctgcttatggtgacaattgtgagattgttaccataaagctattggattggccatccggtgactatcagagctattatatatctttttgttgggtttataccactaagcttgaaagaggttataactctacattacattttaatactgaacaccgcaaaatggtgtcaaagggtgaggaattattcaccggcgtggtgcctatccttgtggaacttgatggagatgtgaacggacacaaattcagtgtatcaggagaaggagaaggagatgcaacatacggaaagctcactcttaaatttatctgcacaacaggaaagctcccggtgccttggcctacacttgtgacaacacttacatacggagtgcaatgcttctcgcgttaccctgatcacatgaaacaacacgatttcttcaagagtgcaatgcctgaaggatacgtgcaagaaagaacaatcttcttcaaggacgatggaaactacaagactcgtgcagaagtgaaatttgaaggagatacacttgtgaacagaatcgaacttaaaggaatcgatttcaaggaggatggaaacatccttggacacaaacttgaatacaactacaactcacacaacgtgtacatcatggcagataaacagaagaatggtatcaaagtgaactttaagattcgccacaacatcgaagatgggt

SEQ ID NO: 39 - DNA, 1639 bp, synthetic construct
  misc_feature 1..1639: note = sequence of circular RNA
  source 1..1639: mol_type = other DNA
aaaatccgttgaccttaaacggtcgtgtgggttcaagtccctccacccccacgccggaaacgcaatagccgaaaaaacaaaaacaaaaaaaacaaaaaaacaaaaaaaaaaccaaaacacattaaaacagcctgtgggttgatcccacccacagggcccactgggcgctagcactctggtatcacggtacctttgtgcgcctgttttatacttcctcccccaactgcaacttagaagtaacacaaaccgatcaacagtcagcgtggcacaccagccacgttttgatcaaacacttctgttaccccggactgagtatcaatagactgctcacgcggttgaaggagaaaacgttcgttatccggccaactacttcgagaaacctagtaacgccatggaagttgtggagtgtttcgctcagcactaccccagtgtagatcaggttgatgagtcaccgcattccccacgggtgaccgtggcggtggctgcgttggcggcctgcccatggggaaacccatgggacgctcttatacagacatggtgcgaagagtctattgagctagttggtagtcctccggcccctgaatgcggctaatcccaactgcggagcatacactctcaagccagagggtagtgtgtcgtaatgggcaactctgcagcggaaccgactactttgggtgtccgtgtttcattttattcctatactggctgcttatggtgacaattgagagattgttaccatatagctattggattggccatccggtgactaacagagctattatatatctttttgttgggtttataccacttagcttgaaagaggttaaaactctacattacattttaatactgaacaccgcaaaatggtgtcaaagggtgaggaattattcaccggcgtggtgcctatccttgtggaacttgatggagatgtgaacggacacaaattcagtgtatcaggagaaggagaaggagatgcaacatacggaaagctcactcttaaatttatctgcacaacaggaaagctcccggtgccttggcctacacttgtgacaacacttacatacggagtgcaatgcttctcgcgttaccctgatcacatgaaacaacacgatttcttcaagagtgcaatgcctgaaggatacgtgcaagaaagaacaatcttcttcaaggacgatggaaactacaagactcgtgcagaagtgaaatttgaaggagatacacttgtgaacagaatcgaacttaaaggaatcgatttcaaggaggatggaaacatccttggacacaaacttgaatacaactacaactcacacaacgtgtacatcatggcagataaacagaagaatggtatcaaagtgaactttaagattcgccacaacatcgaagatggatcagtgcaacttgcagatcactaccaacagaatacgccgataggagatggacctgtgcttcttcctgataaccactacctttcaacacaatcagcactttcaaaggacccaaacgagaagcgagaccacatggtgcttcttgaatttgtgacagcagcaggaatcacacttggaatggatgaactttacaaatgaaaaaaacaaaaaacaaaacggctattatgcgttaccggcgagacgctacggactta

SEQ ID NO: 40 - DNA, 3267 bp, synthetic construct
  misc_feature 1..3267: note = sequence of circular RNA
  source 1..3267: mol_type = other DNA
ctgtgcaacttgcagatcactaccaacagaatacgccgataggagatggacctgtgcttcttcctgataaccactacctttcaacacaatcagcactttcaaaggacccaaacgagaagcgagaccacatggtgcttcttgaatttgtgacagcagcaggaatcacacttggaatggatgaactttacaaaggaagcggagctactaacttcagcctgctgaagcaggctggagacgtggaggagaaccctggacctggaagcggggaggacgccaagaacatcaagaagggccctgcccctttctaccctctggaggacggcaccgccggcgagcagctgcacaaggccatgaagaggtacgccctggtgcctggcaccatcgccttcaccgacgcccacatcgaggtggacatcacctacgccgagtacttcgagatgagcgtgaggctggccgaggccatgaagaggtacggcctgaacaccaaccacaggatcgtggtgtgcagcgagaacagcctgcagttcttcatgcctgtgctgggcgccctgttcatcggcgtggccgtggcccctgccaacgacatctacaacgagagggagctgctgaacagcatgggcatcagccagcctaccgtggtgttcgtgagcaagaagggcctgcagaagatcctgaacgtgcagaagaagctgcctatcatccagaagatcatcatcatggacagcaagaccgactaccagggcttccagagcatgtacaccttcgtgaccagccacctgcctcctggcttcaacgagtacgacttcgtgcctgagagcttcgacagggacaagaccatcgccctgatcatgaacagcagcggcagcaccggcctgcctaagggcgtggccctgcctcacaggaccgcctgcgtgaggttcagccacgccagggaccctatcttcggcaaccagatcatccctgacaccgccatcctgagcgtggtgcctttccaccacggcttcggcatgttcaccaccctgggctacctgatctgcggcttcagggtggtgctgatgtacaggttcgaggaggagctgttcctgaggagcctgcaggactacaagatccagagcgccctgctggtgcctaccctgttcagcttcttcgccaagagcaccctgatcgacaagtacgacctgagcaacctgcacgagatcgccagcggcggcgcccctctgagcaaggaggtgggcgaggccgtggccaagaggttccacctgcctggcatcaggcagggctacggcctgaccgagaccaccagcgccatcctgatcacccctgagggcgacgacaagcctggcgccgtgggcaaggtggtgcctttcttcgaggccaaggtggtggacctggacaccggcaagaccctgggcgtgaaccagaggggcgagctgtgcgtgaggggccctatgatcatgagcggctacgtgaacaaccctgaggccaccaacgccctgatcgacaaggacggctggctgcacagcggcgacatcgcctactgggacgaggacgagcacttcttcatcgtggacaggctgaagagcctgatcaagtacaagggctaccaggtggcccctgccgagctggagagcatcctgctgcagcaccctaacatcttcgacgccggcgtggctggcttgcctgatgacgatgctggagagctgcctgccgccgtggtggtgctggagcacggcaagaccatgaccgagaaggagatcgtggactacgtggccagccaggtgaccaccgccaagaagctgaggggcggcgtggtgttcgtggacgaggtgcctaagggcctgaccggcaagctggacgccaggaagatcagggagatcctgatcaaggccaagaagggcggcaagatcgccgtgtgaggttaaaacagcctgtgggttgatcccacccacagggcccactgggcgctagcactctggtatcacggtacctttgtgcgcctgttttatacttcctcccccaactgcaacttagaagtaacacaaaccgatcaacagtcagcgtggcacaccagccacgttttgatcaaacacttctgttaccccggactgagtatcaatagactgctcacgcggttgaaggagaaaacgttcgttatccggccaactacttcgagaaacctagtaacgccatggaagttgtggagtgtttcgctcagcactaccccagtgtagatcaggttgatgagtcaccgcattccccacgggtgaccgtggcggtggctgcgttggcggcctgcccatggggaaacccatgggacgctcttatacagacatggtgcgaagagtctattgagctagttggtagtcctccggcccctgaatgcggctaatcccaactgcggagcatacactctcaagccagagggtagtgtgtcgtaatgggcaactctgcagcggaaccgactactttgggtgtccgtgtttcattttattcctatactggctgcttatggtgacaattgagagattgttaccatatagctattggattggccatccggtgactaacagagctattatatatctttttgttgggtttataccacttagcttgaaagaggttaaaactctacattacattttaatactgaacaccgcaaaggagccaccatgggctccggcgagggcaggggaagtcttctaacatgcggggacgtggaggaaaatcccggcccaggctccggcgtgtcaaagggtgaggaattattcaccggcgtggtgcctatccttgtggaacttgatggagatgtgaacggacacaaattcagtgtatcaggagaaggagaaggagatgcaacatacggaaagctcactcttaaatttatctgcacaacaggaaagctcccggtgccttggcctacacttgtgacaacacttacatacggagtgcaatgcttctcgcgttaccctgatcacatgaaacaacacgatttcttcaagagtgcaatgcctgaaggatacgtgcaagaaagaacaatcttcttcaaggacgatggaaactacaagactcgtgcagaagtgaaatttgaaggagatacacttgtgaacagaatcgaacttaaaggaatcgatttcaaggaggatggaaacatccttggacacaaacttgaatacaactacaactcacacaacgtgtacatcatggcagataaacagaagaatggtatcaaagtgaactttaagattcgccacaacatcgaagatgggt

SEQ ID NO: 41 - DNA, 3752 bp, synthetic construct
  misc_feature 1..3752: note = sequence of circular RNA
  source 1..3752: mol_type = other DNA
ctgtgcaacttgcagatcactaccaacagaatacgccgataggagatggacctgtgcttcttcctgataaccactacctttcaacacaatcagcactttcaaaggacccaaacgagaagcgagaccacatggtgcttcttgaatttgtgacagcagcaggaatcacacttggaatggatgaactttacaaatgaacgttactggccgaagccgcttggaacaaggccggtgtgcgtttgtctatatgttattttccaccatattgccgtcttttggcaatgtgagggcccggaaacctggccctgtcttcttgacgagcattcctaggggtctttcccctctcgccaaaggaatgcaaggtctgttgaatgtcgtgaaggaagcagttcctctggaagcttcttgtagacaaacaacgtctgtagcgaccctttgcaggcagcggaaccccccacctggcgacaggtgcctctgcggccaaaagccacgtgtatacgatacacctgcaaaggcggcacaaccccagtgccacgttgtgagttggatagttgtggaaagagtcaaatggctctcctcaagcgtattcaacaaggggctgaaggatgcccagaaggtaccccattgtatgggatctgatctggggcctcggtgcacatgctttacatgtgttcagtcgaggttaaaaaacgtccaggccccccgaaccacggggacgtggttttcctttgaaaaacacgatgataatatggccacaaccatggaggacgccaagaacatcaagaagggccctgcccctttctaccctctggaggacggcaccgccggcgagcagctgcacaaggccatgaagaggtacgccctggtgcctggcaccatcgccttcaccgacgcccacatcgaggtggacatcacctacgccgagtacttcgagatgagcgtgaggctggccgaggccatgaagaggtacggcctgaacaccaaccacaggatcgtggtgtgcagcgagaacagcctgcagttcttcatgcctgtgctgggcgccctgttcatcggcgtggccgtggcccctgccaacgacatctacaacgagagggagctgctgaacagcatgggcatcagccagcctaccgtggtgttcgtgagcaagaagggcctgcagaagatcctgaacgtgcagaagaagctgcctatcatccagaagatcatcatcatggacagcaagaccgactaccagggcttccagagcatgtacaccttcgtgaccagccacctgcctcctggcttcaacgagtacgacttcgtgcctgagagcttcgacagggacaagaccatcgccctgatcatgaacagcagcggcagcaccggcctgcctaagggcgtggccctgcctcacaggaccgcctgcgtgaggttcagccacgccagggaccctatcttcggcaaccagatcatccctgacaccgccatcctgagcgtggtgcctttccaccacggcttcggcatgttcaccaccctgggctacctgatctgcggcttcagggtggtgctgatgtacaggttcgaggaggagctgttcctgaggagcctgcaggactacaagatccagagcgccctgctggtgcctaccctgttcagcttcttcgccaagagcaccctgatcgacaagtacgacctgagcaacctgcacgagatcgccagcggcggcgcccctctgagcaaggaggtgggcgaggccgtggccaagaggttccacctgcctggcatcaggcagggctacggcctgaccgagaccaccagcgccatcctgatcacccctgagggcgacgacaagcctggcgccgtgggcaaggtggtgcctttcttcgaggccaaggtggtggacctggacaccggcaagaccctgggcgtgaaccagaggggcgagctgtgcgtgaggggccctatgatcatgagcggctacgtgaacaaccctgaggccaccaacgccctgatcgacaaggacggctggctgcacagcggcgacatcgcctactgggacgaggacgagcacttcttcatcgtggacaggctgaagagcctgatcaagtacaagggctaccaggtggcccctgccgagctggagagcatcctgctgcagcaccctaacatcttcgacgccggcgtggctggcttgcctgatgacgatgctggagagctgcctgccgccgtggtggtgctggagcacggcaagaccatgaccgagaaggagatcgtggactacgtggccagccaggtgaccaccgccaagaagctgaggggcggcgtggtgttcgtggacgaggtgcctaagggcctgaccggcaagctggacgccaggaagatcagggagatcctgatcaaggccaagaagggcggcaagatcgccgtgtgaggttaaaacagcctgtgggttgatcccacccacagggcccactgggcgctagcactctggtatcacggtacctttgtgcgcctgttttatacttcctcccccaactgcaacttagaagtaacacaaaccgatcaacagtcagcgtggcacaccagccacgttttgatcaaacacttctgttaccccggactgagtatcaatagactgctcacgcggttgaaggagaaaacgttcgttatccggccaactacttcgagaaacctagtaacgccatggaagttgtggagtgtttcgctcagcactaccccagtgtagatcaggttgatgagtcaccgcattccccacgggtgaccgtggcggtggctgcgttggcggcctgcccatggggaaacccatgggacgctcttatacagacatggtgcgaagagtctattgagctagttggtagtcctccggcccctgaatgcggctaatcccaactgcggagcatacactctcaagccagagggtagtgtgtcgtaatgggcaactctgcagcggaaccgactactttgggtgtccgtgtttcattttattcctatactggctgcttatggtgacaattgagagattgttaccatatagctattggattggccatccggtgactaacagagctattatatatctttttgttgggtttataccacttagcttgaaagaggttaaaactctacattacattttaatactgaacaccgcaaaatgggctccggcgagggcaggggaagtcttctaacatgcggggacgtggaggaaaatcccggcccaggctccggcgtgtcaaagggtgaggaattattcaccggcgtggtgcctatccttgtggaacttgatggagatgtgaacggacacaaattcagtgtatcaggagaaggagaaggagatgcaacatacggaaagctcactcttaaatttatctgcacaacaggaaagctcccggtgccttggcctacacttgtgacaacacttacatacggagtgcaatgcttctcgcgttaccctgatcacatgaaacaacacgatttcttcaagagtgcaatgcctgaaggatacgtgcaagaaagaacaatcttcttcaaggacgatggaaactacaagactcgtgcagaagtgaaatttgaaggagatacacttgtgaacagaatcgaacttaaaggaatcgatttcaaggaggatggaaacatccttggacacaaacttgaatacaactacaactcacacaacgtgtacatcatggcagataaacagaagaatggtatcaaagtgaactttaagattcgccacaacatcgaagatgggt

SEQ ID NO: 42 - DNA, 20 bp, synthetic construct
  misc_feature 1..20: note = primer sequence
  source 1..20: mol_type = other DNA
tgggaggattctgcattacc

SEQ ID NO: 43 - DNA, 18 bp, synthetic construct
  misc_feature 1..18: note = primer sequence
  source 1..18: mol_type = other DNA
cagcatcgctggttgaga

SEQ ID NO: 44 - DNA, 20 bp, synthetic construct
  misc_feature 1..20: note = primer sequence
  source 1..20: mol_type = other DNA
ctcccggcacagaagtgtat

SEQ ID NO: 45 - DNA, 20 bp, synthetic construct
  misc_feature 1..20: note = primer sequence
  source 1..20: mol_type = other DNA
cttcctctgcctctggtttg

SEQ ID NO: 46 - DNA, 20 bp, synthetic construct
  misc_feature 1..20: note = primer sequence
  source 1..20: mol_type = other DNA
ccatctctgtcctccatgag

SEQ ID NO: 47 - DNA, 20 bp, synthetic construct
  misc_feature 1..20: note = primer sequence
  source 1..20: mol_type = other DNA
atttctgctctgacaacctc

SEQ ID NO: 48 - DNA, 20 bp, synthetic construct
  misc_feature 1..20: note = primer sequence
  source 1..20: mol_type = other DNA
tgcaaaatgggacagaaaga

SEQ ID NO: 49 - DNA, 20 bp, synthetic construct
  misc_feature 1..20: note = primer sequence
  source 1..20: mol_type = other DNA
tgattcagaagcgagtgtgc

SEQ ID NO: 50 - DNA, 20 bp, synthetic construct
  misc_feature 1..20: note = primer sequence
  source 1..20: mol_type = other DNA
accaaatacaggagccatgc

SEQ ID NO: 51 - DNA, 20 bp, synthetic construct
  misc_feature 1..20: note = primer sequence
  source 1..20: mol_type = other DNA
gcgatttccttcttttgcag

SEQ ID NO: 52 - DNA, 20 bp, synthetic construct
  misc_feature 1..20: note = primer sequence
  source 1..20: mol_type = other DNA
cgtctcctaccagaccaagg

SEQ ID NO: 53 - DNA, 20 bp, synthetic construct
  misc_feature 1..20: note = primer sequence
  source 1..20: mol_type = other DNA
ccaaagtagacctgcccaga

SEQ ID NO: 54 - DNA, 20 bp, synthetic construct
  misc_feature 1..20: note = primer sequence
  source 1..20: mol_type = other DNA
tacccccaggagaagattcc

SEQ ID NO: 55 - DNA, 20 bp, synthetic construct
  misc_feature 1..20: note = primer sequence
  source 1..20: mol_type = other DNA
gccatctttggaaggttcag

SEQ ID NO: 56 - DNA, 2514 bp, synthetic construct
  misc_feature 1..2514: note = sequence of circular RNA
  source 1..2514: mol_type = other DNA
ttaaaacagcctgtgggttgatcccacccacagggcccactgggcgctagcactctggtatcacggtacctttgtgcgcctgttttatacttcctcccccaactgcaacttagaagtaacacaaaccgatcaacagtcagcgtggcacaccagccacgttttgatcaaacacttctgttaccccggactgagtatcaatagactgctcacgcggttgaaggagaaaacgttcgttatccggccaactacttcgagaaacctagtaacgccatggaagttgtggagtgtttcgctcagcactaccccagtgtagatcaggttgatgagtcaccgcattccccacgggtgaccgtggcggtggctgcgttggcggcctgcccatggggaaacccatgggacgctcttatacagacatggtgcgaagagtctattgagctagttggtagtcctccggcccctgaatgcggctaatcccaactgcggagcatacactctcaagccagagggtagtgtgtcgtaatgggcaactctgcagcggaaccgactactttgggtgtccgtgtttcattttattcctatactggctgcttatggtgacaattgagagattgttaccatatagctattggattggccatccggtgactaacagagctattatatatctttttgttgggtttataccacttagcttgaaagaggttaaaactctacattacattttaatactgaacaccgcaaaatggaggacgccaagaacatcaagaagggccctgcccctttctaccctctggaggacggcaccgccggcgagcagctgcacaaggccatgaagaggtacgccctggtgcctggcaccatcgccttcaccgacgcccacatcgaggtggacatcacctacgccgagtacttcgagatgagcgtgaggctggccgaggccatgaagaggtacggcctgaacaccaaccacaggatcgtggtgtgcagcgagaacagcctgcagttcttcatgcctgtgctgggcgccctgttcatcggcgtggccgtggcccctgccaacgacatctacaacgagagggagctgctgaacagcatgggcatcagccagcctaccgtggtgttcgtgagcaagaagggcctgcagaagatcctgaacgtgcagaagaagctgcctatcatccagaagatcatcatcatggacagcaagaccgactaccagggcttccagagcatgtacaccttcgtgaccagccacctgcctcctggcttcaacgagtacgacttcgtgcctgagagcttcgacagggacaagaccatcgccctgatcatgaacagcagcggcagcaccggcctgcctaagggcgtggccctgcctcacaggaccgcctgcgtgaggttcagccacgccagggaccctatcttcggcaaccagatcatccctgacaccgccatcctgagcgtggtgcctttccaccacggcttcggcatgttcaccaccctgggctacctgatctgcggcttcagggtggtgctgatgtacaggttcgaggaggagctgttcctgaggagcctgcaggactacaagatccagagcgccctgctggtgcctaccctgttcagcttcttcgccaagagcaccctgatcgacaagtacgacctgagcaacctgcacgagatcgccagcggcggcgcccctctgagcaaggaggtgggcgaggccgtggccaagaggttccacctgcctggcatcaggcagggctacggcctgaccgagaccaccagcgccatcctgatcacccctgagggcgacgacaagcctggcgccgtgggcaaggtggtgcctttcttcgaggccaaggtggtggacctggacaccggcaagaccctgggcgtgaaccagaggggcgagctgtgcgtgaggggccctatgatcatgagcggctacgtgaacaaccctgaggccaccaacgccctgatcgacaaggacggctggctgcacagcggcgacatcgcctactgggacgaggacgagcacttcttcatcgtggacaggctgaagagcctgatcaagtacaagggctaccaggtggcccctgccgagctggagagcatcctgctgcagcaccctaacatcttcgacgccggcgtggctggcttgcctgatgacgatgctggagagctgcctgccgccgtggtggtgctggagcacggcaagaccatgaccgagaaggagatcgtggactacgtggccagccaggtgaccaccgccaagaagctgaggggcggcgtggtgttcgtggacgaggtgcctaagggcctgaccggcaagctggacgccaggaagatcagggagatcctgatcaaggccaagaagggcggcaagatcgccgtgtgatgataataggctggagcctcggtggccatgcttcttgccccttgggcctccccccagcccctcctccccttcctgcacccgtacccccgtggtctttgaataaagtctgagtgggcggc

SEQ ID NO: 57 - DNA, 2536 bp, synthetic construct
  misc_feature 1..2536: note = sequence of circular RNA
  source 1..2536: mol_type = other DNA
ttaaaacagcctgtgggttgatcccacccacagggcccactgggcgctagcactctggtatcacggtacctttgtgcgcctgttttatacttcctcccccaactgcaacttagaagtaacacaaaccgatcaacagtcagcgtggcacaccagccacgttttgatcaaacacttctgttaccccggactgagtatcaatagactgctcacgcggttgaaggagaaaacgttcgttatccggccaactacttcgagaaacctagtaacgccatggaagttgtggagtgtttcgctcagcactaccccagtgtagatcaggttgatgagtcaccgcattccccacgggtgaccgtggcggtggctgcgttggcggcctgcccatggggaaacccatgggacgctcttatacagacatggtgcgaagagtctattgagctagttggtagtcctccggcccctgaatgcggctaatcccaactgcggagcatacactctcaagccagagggtagtgtgtcgtaatgggcaactctgcagcggaaccgactactttgggtgtccgtgtttcattttattcctatactggctgcttatggtgacaattgagagattgttaccatatagctattggattggccatccggtgactaacagagctattatatatctttttgttgggtttataccacttagcttgaaagaggttaaaactctacattacattttaatactgaacaccgcaaaatggaggacgccaagaacatcaagaagggccctgcccctttctaccctctggaggacggcaccgccggcgagcagctgcacaaggccatgaagaggtacgccctggtgcctggcaccatcgccttcaccgacgcccacatcgaggtggacatcacctacgccgagtacttcgagatgagcgtgaggctggccgaggccatgaagaggtacggcctgaacaccaaccacaggatcgtggtgtgcagcgagaacagcctgcagttcttcatgcctgtgctgggcgccctgttcatcggcgtggccgtggcccctgccaacgacatctacaacgagagggagctgctgaacagcatgggcatcagccagcctaccgtggtgttcgtgagcaagaagggcctgcagaagatcctgaacgtgcagaagaagctgcctatcatccagaagatcatcatcatggacagcaagaccgactaccagggcttccagagcatgtacaccttcgtgaccagccacctgcctcctggcttcaacgagtacgacttcgtgcctgagagcttcgacagggacaagaccatcgccctgatcatgaacagcagcggcagcaccggcctgcctaagggcgtggccctgcctcacaggaccgcctgcgtgaggttcagccacgccagggaccctatcttcggcaaccagatcatccctgacaccgccatcctgagcgtggtgcctttccaccacggcttcggcatgttcaccaccctgggctacctgatctgcggcttcagggtggtgctgatgtacaggttcgaggaggagctgttcctgaggagcctgcaggactacaagatccagagcgccctgctggtgcctaccctgttcagcttcttcgccaagagcaccctgatcgacaagtacgacctgagcaacctgcacgagatcgccagcggcggcgcccctctgagcaaggaggtgggcgaggccgtggccaagaggttccacctgcctggcatcaggcagggctacggcctgaccgagaccaccagcgccatcctgatcacccctgagggcgacgacaagcctggcgccgtgggcaaggtggtgcctttcttcgaggccaaggtggtggacctggacaccggcaagaccctgggcgtgaaccagaggggcgagctgtgcgtgaggggccctatgatcatgagcggctacgtgaacaaccctgaggccaccaacgccctgatcgacaaggacggctggctgcacagcggcgacatcgcctactgggacgaggacgagcacttcttcatcgtggacaggctgaagagcctgatcaagtacaagggctaccaggtggcccctgccgagctggagagcatcctgctgcagcaccctaacatcttcgacgccggcgtggctggcttgcctgatgacgatgctggagagctgcctgccgccgtggtggtgctggagcacggcaagaccatgaccgagaaggagatcgtggactacgtggccagccaggtgaccaccgccaagaagctgaggggcggcgtggtgttcgtggacgaggtgcctaagggcctgaccggcaagctggacgccaggaagatcagggagatcctgatcaaggccaagaagggcggcaagatcgccgtgtgatgataataggctggagcctcggtggccatgcttcttgccccttgggcctccccccagcccctcctccccttcctgcacccgtaccccccaaacaccattgtcacactccagtggtctttgaataaagtctgagtgggcggc

SEQ ID NO: 58 - DNA, 2580 bp, synthetic construct
  misc_feature 1..2580: note = sequence of circular RNA
  source 1..2580: mol_type = other DNA
ttaaaacagcctgtgggttgatcccacccacagggcccactgggcgctagcactctggtatcacggtacctttgtgcgcctgttttatacttcctcccccaactgcaacttagaagtaacacaaaccgatcaacagtcagcgtggcacaccagccacgttttgatcaaacacttctgttaccccggactgagtatcaatagactgctcacgcggttgaaggagaaaacgttcgttatccggccaactacttcgagaaacctagtaacgccatggaagttgtggagtgtttcgctcagcactaccccagtgtagatcaggttgatgagtcaccgcattccccacgggtgaccgtggcggtggctgcgttggcggcctgcccatggggaaacccatgggacgctcttatacagacatggtgcgaagagtctattgagctagttggtagtcctccggcccctgaatgcggctaatcccaactgcggagcatacactctcaagccagagggtagtgtgtcgtaatgggcaactctgcagcggaaccgactactttgggtgtccgtgtttcattttattcctatactggctgcttatggtgacaattgagagattgttaccatatagctattggattggccatccggtgactaacagagctattatatatctttttgttgggtttataccacttagcttgaaagaggttaaaactctacattacattttaatactgaacaccgcaaaatggaggacgccaagaacatcaagaagggccctgcccctttctaccctctggaggacggcaccgccggcgagcagctgcacaaggccatgaagaggtacgccctggtgcctggcaccatcgccttcaccgacgcccacatcgaggtggacatcacctacgccgagtacttcgagatgagcgtgaggctggccgaggccatgaagaggtacggcctgaacaccaaccacaggatcgtggtgtgcagcgagaacagcctgcagttcttcatgcctgtgctgggcgccctgttcatcggcgtggccgtggcccctgccaacgacatctacaacgagagggagctgctgaacagcatgggcatcagccagcctaccgtggtgttcgtgagcaagaagggcctgcagaagatcctgaacgtgcagaagaagctgcctatcatccagaagatcatcatcatggacagcaagaccgactaccagggcttccagagcatgtacaccttcgtgaccagccacctgcctcctggcttcaacgagtacgacttcgtgcctgagagcttcgacagggacaagaccatcgccctgatcatgaacagcagcggcagcaccggcctgcctaagggcgtggccctgcctcacaggaccgcctgcgtgaggttcagccacgccagggaccctatcttcggcaaccagatcatccctgacaccgccatcctgagcgtggtgcctttccaccacggcttcggcatgttcaccaccctgggctacctgatctgcggcttcagggtggtgctgatgtacaggttcgaggaggagctgttcctgaggagcctgcaggactacaagatccagagcgccctgctggtgcctaccctgttcagcttcttcgccaagagcaccctgatcgacaagtacgacctgagcaacctgcacgagatcgccagcggcggcgcccctctgagcaaggaggtgggcgaggccgtggccaagaggttccacctgcctggcatcaggcagggctacggcctgaccgagaccaccagcgccatcctgatcacccctgagggcgacgacaagcctggcgccgtgggcaaggtggtgcctttcttcgaggccaaggtggtggacctggacaccggcaagaccctgggcgtgaaccagaggggcgagctgtgcgtgaggggccctatgatcatgagcggctacgtgaacaaccctgaggccaccaacgccctgatcgacaaggacggctggctgcacagcggcgacatcgcctactgggacgaggacgagcacttcttcatcgtggacaggctgaagagcctgatcaagtacaagggctaccaggtggcccctgccgagctggagagcatcctgctgcagcaccctaacatcttcgacgccggcgtggctggcttgcctgatgacgatgctggagagctgcctgccgccgtggtggtgctggagcacggcaagaccatgaccgagaaggagatcgtggactacgtggccagccaggtgaccaccgccaagaagctgaggggcggcgtggtgttcgtggacgaggtgcctaagggcctgaccggcaagctggacgccaggaagatcagggagatcctgatcaaggccaagaagggcggcaagatcgccgtgtgatgataatagcaaacaccattgtcacactccagctggagcctcggtggccatgcttcttgccccttgggcccaaacaccattgtcacactccatccccccagcccctcctccccttcctgcacccgtaccccccaaacaccattgtcacactccagtggtctttgaataaagtctgagtgggcggc

SEQ ID NO: 59 - DNA, 2754 bp, synthetic construct
  misc_feature 1..2754: note = sequence of circular RNA
  source 1..2754: mol_type = other DNA
ttaaaacagcctgtgggttgatcccacccacagggcccactgggcgctagcactctggtatcacggtacctttgtgcgcctgttttatacttcctcccccaactgcaacttagaagtaacacaaaccgatcaacagtcagcgtggcacaccagccacgttttgatcaaacacttctgttaccccggactgagtatcaatagactgctcacgcggttgaaggagaaaacgttcgttatccggccaactacttcgagaaacctagtaacgccatggaagttgtggagtgtttcgctcagcactaccccagtgtagatcaggttgatgagtcaccgcattccccacgggtgaccgtggcggtggctgcgttggcggcctgcccatggggaaacccatgggacgctcttatacagacatggtgcgaagagtctattgagctagttggtagtcctccggcccctgaatgcggctaatcccaactgcggagcatacactctcaagccagagggtagtgtgtcgtaatgggcaactctgcagcggaaccgactactttgggtgtccgtgtttcattttattcctatactggctgcttatggtgacaattgagagattgttaccatatagctattggattggccatccggtgactaacagagctattatatatctttttgttgggtttataccacttagcttgaaagaggttaaaactctacattacattttaatactgaacaccgcaaaatggaggacgccaagaacatcaagaagggccctgcccctttctaccctctggaggacggcaccgccggcgagcagctgcacaaggccatgaagaggtacgccctggtgcctggcaccatcgccttcaccgacgcccacatcgaggtggacatcacctacgccgagtacttcgagatgagcgtgaggctggccgaggccatgaagaggtacggcctgaacaccaaccacaggatcgtggtgtgcagcgagaacagcctgcagttcttcatgcctgtgctgggcgccctgttcatcggcgtggccgtggcccctgccaacgacatctacaacgagagggagctgctgaacagcatgggcatcagccagcctaccgtggtgttcgtgagcaagaagggcctgcagaagatcctgaacgtgcagaagaagctgcctatcatccagaagatcatcatcatggacagcaagaccgactaccagggcttccagagcatgtacaccttcgtgaccagccacctgcctcctggcttcaacgagtacgacttcgtgcctgagagcttcgacagggacaagaccatcgccctgatcatgaacagcagcggcagcaccggcctgcctaagggcgtggccctgcctcacaggaccgcctgcgtgaggttcagccacgccagggaccctatcttcggcaaccagatcatccctgacaccgccatcctgagcgtggtgcctttccaccacggcttcggcatgttcaccaccctgggctacctgatctgcggcttcagggtggtgctgatgtacaggttcgaggaggagctgttcctgaggagcctgcaggactacaagatccagagcgccctgctggtgcctaccctgttcagcttcttcgccaagagcaccctgatcgacaagtacgacctgagcaacctgcacgagatcgccagcggcggcgcccctctgagcaaggaggtgggcgaggccgtggccaagaggttccacctgcctggcatcaggcagggctacggcctgaccgagaccaccagcgccatcctgatcacccctgagggcgacgacaagcctggcgccgtgggcaaggtggtgcctttcttcgaggccaaggtggtggacctggacaccggcaagaccctgggcgtgaaccagaggggcgagctgtgcgtgaggggccctatgatcatgagcggctacgtgaacaaccctgaggccaccaacgccctgatcgacaaggacggctggctgcacagcggcgacatcgcctactgggacgaggacgagcacttcttcatcgtggacaggctgaagagcctgatcaagtacaagggctaccaggtggcccctgccgagctggagagcatcctgctgcagcaccctaacatcttcgacgccggcgtggctggcttgcctgatgacgatgctggagagctgcctgccgccgtggtggtgctggagcacggcaagaccatgaccgagaaggagatcgtggactacgtggccagccaggtgaccaccgccaagaagctgaggggcggcgtggtgttcgtggacgaggtgcctaagggcctgaccggcaagctggacgccaggaagatcagggagatcctgatcaaggccaagaagggcggcaagatcgccgtgtgatgataatagatgcggccgccgaccagaatcatgcaagtgcgtaagatagtcgcgggtcggcggccgcatgctggagcctcggtggccatgcttcttgccccttgggccatgcggccgccgaccagaatcatgcaagtgcgtaagatagtcgcgggtcggcggccgcattccccccagcccctcatgcggccgccgaccagaatcatgcaagtgcgtaagatagtcgcgggtcggcggccgcatctccccttcctgcacccgtacccccatgcggccgccgaccagaatcatgcaagtgcgtaagatagtcgcgggtcggcggccgcatgtggtctttgaataaagtctgagtgggcggc

SEQ ID NO: 60 - protein, 4 aa, synthetic construct
  REGION 1..4: note = sequence of amino acid unit
MVSK

SEQ ID NO: 61 - protein, 4 aa, synthetic construct
  REGION 1..4: note = sequence of amino acid unit
VSKG

SEQ ID NO: 62 - protein, 4 aa, synthetic construct
  REGION 1..4: note = sequence of amino acid unit
SKGE

SEQ ID NO: 63 - protein, 4 aa, synthetic construct
  REGION 1..4: note = sequence of amino acid unit
ELYK

SEQ ID NO: 64 - skipped

SEQ ID NO: 65 - DNA, 12 bp, synthetic construct
  misc_feature 1..12: note = codon sequence
  source 1..12: mol_type = other DNA
ttttcggtctct

SEQ ID NO: 66 - DNA, 12 bp, synthetic construct
  misc_feature 1..12: note = codon sequence
  source 1..12: mol_type = other DNA
attttggtcgag

SEQ ID NO: 67 - DNA, 12 bp, synthetic construct
  misc_feature 1..12: note = codon sequence
  source 1..12: mol_type = other DNA
actttggtcaat

SEQ ID NO: 68 - DNA, 12 bp, synthetic construct
  misc_feature 1..12: note = codon sequence
  source 1..12: mol_type = other DNA
ggttcggtccag

SEQ ID NO: 69 - DNA, 12 bp, synthetic construct
  misc_feature 1..12: note = codon sequence
  source 1..12: mol_type = other DNA
ttttcggtcagt

SEQ ID NO: 70 - DNA, 12 bp, synthetic construct
  misc_feature 1..12: note = codon sequence
  source 1..12: mol_type = other DNA
actggggtcgtt

SEQ ID NO: 71 - DNA, 12 bp, synthetic construct
  misc_feature 1..12: note = codon sequence
  source 1..12: mol_type = other DNA
tatggggtccag

SEQ ID NO: 72 - skipped

SEQ ID NO: 73 - DNA, 12 bp, synthetic construct
  misc_feature 1..12: note = codon sequence
  source 1..12: mol_type = other DNA
attctgggtcat

SEQ ID NO: 74 - DNA, 12 bp, synthetic construct
  misc_feature 1..12: note = codon sequence
  source 1..12: mol_type = other DNA
actctgggtatg

SEQ ID NO: 75 - DNA, 12 bp, synthetic construct
  misc_feature 1..12: note = codon sequence
  source 1..12: mol_type = other DNA
acgctgggtatg

SEQ ID NO: 76 - DNA, 12 bp, synthetic construct
  misc_feature 1..12: note = codon sequence
  source 1..12: mol_type = other DNA
atcctgggtcat

SEQ ID NO: 77 - DNA, 12 bp, synthetic construct
  misc_feature 1..12: note = codon sequence
  source 1..12: mol_type = other DNA
accctgggtatg

SEQ ID NO: 78 - DNA, 12 bp, synthetic construct
  misc_feature 1..12: note = codon sequence
  source 1..12: mol_type = other DNA
atactgggtcat

SEQ ID NO: 79 - DNA, 12 bp, synthetic construct
  misc_feature 1..12: note = codon sequence
  source 1..12: mol_type = other DNA
acactgggtatg

SEQ ID NO: 80 - DNA, 13 bp, synthetic construct
  misc_feature 1..13: note = sequence of ribozyme recognition site
  source 1..13: mol_type = other DNA
acgtcttaaccaa